European Patent Specification EP 4 105 317 B1, published February 25, 2026. Title: Bacillus subtilis JCK-1398 strain having induced resistance in various plant, composition for controlling pine wilt disease comprising the same and method used therein. Applicant: INDUSTRY FOUNDATION OF CHONNAM NATIONAL UNIVERSITY National Institute of Forest Science Pusan National University Industry-University Cooperation Foundation. The sequence listing filed with the application follows.

SEQUENCE LISTING (33 sequences)

SEQ ID NO: 1 - DNA, 20 bp, Artificial Sequence
  PR-1b family For
tgccccttcaggtaaatcgt

SEQ ID NO: 2 - DNA, 21 bp, Artificial Sequence
  PR-1b family Rev
gcgggtcgtagttgcagataa

SEQ ID NO: 3 - DNA, 20 bp, Artificial Sequence
  PR-2 family For
cgacaacattcgccccttct

SEQ ID NO: 4 - DNA, 20 bp, Artificial Sequence
  PR-2 family Rev
ctgcagcgcggtttgaatat

SEQ ID NO: 5 - DNA, 19 bp, Artificial Sequence
  PR-3 family class 1 For
acctacagcgcttcattgc

SEQ ID NO: 6 - DNA, 20 bp, Artificial Sequence
  PR-3 family class 1 Rev
tgtggtttcatgcgacgttt

SEQ ID NO: 7 - DNA, 21 bp, Artificial Sequence
  PR-3 family class 4 For
ccatcgaagcccaggtaattt

SEQ ID NO: 8 - DNA, 22 bp, Artificial Sequence
  PR-3 family class 4 Rev
agccgggaagcaatattatggt

SEQ ID NO: 9 - DNA, 21 bp, Artificial Sequence
  PR-4 family For
ccccgttactgtcaattgcat

SEQ ID NO: 10 - DNA, 20 bp, Artificial Sequence
  PR-4 family Rev
aaagcgtgacggtgcgtatt

SEQ ID NO: 11 - DNA, 23 bp, Artificial Sequence
  PR-5 family For
gaaccagtgcccatacacagtct

SEQ ID NO: 12 - DNA, 21 bp, Artificial Sequence
  PR-5 family Rev
cctgcggcaacgttaaaagtc

SEQ ID NO: 13 - DNA, 20 bp, Artificial Sequence
  PR-9 family For
acaccaccgtgctggacatt

SEQ ID NO: 14 - DNA, 20 bp, Artificial Sequence
  PR-9 family Rev
gtgcgggagtcggtgtagag

SEQ ID NO: 15 - DNA, 21 bp, Artificial Sequence
  PR-10 family For
tgtctcaagtggaggcaagga

SEQ ID NO: 16 - DNA, 22 bp, Artificial Sequence
  PR-10 family Rev
aagcgacaatttcaggcaaaac

SEQ ID NO: 17 - DNA, 20 bp, Artificial Sequence
  Antimicrobial peptide For
gcgttgctcatacccgtttt

SEQ ID NO: 18 - DNA, 22 bp, Artificial Sequence
  Antimicrobial peptide Rev
gcagcacttagcactggatgaa

SEQ ID NO: 19 - DNA, 20 bp, Artificial Sequence
  Cytochrome P450 For
aacatgtcctgcagcacgaa

SEQ ID NO: 20 - DNA, 20 bp, Artificial Sequence
  Cytochrome P450 Rev
gtgcaccgcaagtaaaccaa

SEQ ID NO: 21 - DNA, 22 bp, Artificial Sequence
  Extensin For
cgaatgtaattccgaagttgca

SEQ ID NO: 22 - DNA, 20 bp, Artificial Sequence
  Extensin Rev
ccatcccaaaccaccagtct

SEQ ID NO: 23 - DNA, 23 bp, Artificial Sequence
  Hydroxyproline-rich glycoprotein precursor For
gagaaactggcaccgtcttagga

SEQ ID NO: 24 - DNA, 20 bp, Artificial Sequence
  Hydroxyproline-rich glycoprotein precursor Rev
acctccccctccatctcaca

SEQ ID NO: 25 - DNA, 20 bp, Artificial Sequence
  Metallothionein-like protein For
tcaggctgctgcgttatttg

SEQ ID NO: 26 - DNA, 21 bp, Artificial Sequence
  Metallothionein-like protein Rev
tgtcagcgcagtcacaatttg

SEQ ID NO: 27 - DNA, 19 bp, Artificial Sequence
  Xyloglucan endotransglycosylase For
tctgcgcccctacttttcc

SEQ ID NO: 28 - DNA, 20 bp, Artificial Sequence
  Xyloglucan endotransglycosylase Rev
agctgggcgattgatcatgt

SEQ ID NO: 29 - DNA, 20 bp, Artificial Sequence
  Elongation factor-1 alpha For
gggaagccacccaaagtttt

SEQ ID NO: 30 - DNA, 20 bp, Artificial Sequence
  Elongation factor-1 alpha Rev
tacatgggaagacgccgaat

SEQ ID NO: 31 - DNA, 24 bp, Artificial Sequence
  gyrA For
cagtcaggaaatgcgtacgtcctt

SEQ ID NO: 32 - DNA, 24 bp, Artificial Sequence
  gyrA Rev
caaggtaatgctccaggcattgct

SEQ ID NO: 33 - DNA, 856 bp, Artificial Sequence
  Bacillus subtilis JCK-1398 strain gyrA sequence
gatgtttgtagagcagtttgtttgtacagattgtttaagatgacattcgcattggcatcgcgtctgatttcaatgacaattctcatacctgtacgatctgactcatcacgcagatctgtgataccctctatctttttgtcccttacgagatcagcaattttctcaattaatttcgccttatttacttggtaaggtaactctgtaacgataattctttctttacccgaagatgtttgttcgatctcagcttttgcccggatcgtgatagagcctcggcctgattcgtatgctttccggataccgctgcggcccaagatttgacccgcagtcgggaaatcaggtcctggaatgacttccataagctctggaatggtaatgtccggattctcactgacagcaagtactccgtcaatgatttctcccagctggtgcggaggaatgtttgttgccatacctaccgcaatgccggcagcaccgttcacgagcagattcgggaaccttgaaggcataacgacaggttctctttctgacccgtcatagttatcctggtaatcgattgtgtcttttgtgatgtcacgaagaatctccattgagattttagacattcttgcttctgtataacgcatggccgccgctgagtctccgtcaacagaaccgaagtttccgtgaccgtcaacgagcatataacggtagttgaaatcctgagccattctgaccatggattcatataccgctgaatcaccgtgcgggtggtatttcccgataacttctccaacgatacgcgcggattttttataaggcttgtcacttgtcatgcctaaatcattcattgcatacaaaatccgtctatgaactg